European Patent Application EP 4 406 975 A2, published July 31, 2024. Title: COMPOUND HAVING AFFINITY SUBSTANCE TO ANTIBODY AND BIOORTHOGONAL FUNCTIONAL GROUP, OR SALT THEREOF. Applicant: Ajinomoto Co., Inc. Application EP 24163998.8, filed June 14, 2019. The sequence listing filed with the application follows.

SEQUENCE LISTING (108 sequences)

SEQ ID NO: 1 - protein, 230 aa, synthetic construct
  REGION 1..230: note = Fc region of human IgG1
  REGION 18..19: note = misc_feature - Xaa can be any naturally occurring amino acid
  SITE 21: note = misc_feature - Xaa can be any naturally occurring amino acid
  SITE 140: note = misc_feature - Xaa can be any naturally occurring amino acid
  SITE 142: note = misc_feature - Xaa can be any naturally occurring amino acid
  SITE 177: note = misc_feature - Xaa can be any naturally occurring amino acid
PKSCDKTHTCPPCPAPEXXGXPSVFLFPPKPKDTLMISRTPEVTCVVVDVSHEDPEVKFNWYVDGVEVHNAKTKPREEQYDSTYRVVSVLTVLHQDWLNGKEYKCKVSNKALPAPIEKTISKAKGQPREPQVYTLPPSRXEXTKNQVSLTCLVKGFYPSDIAVEWESNGQPENNYKXTPPVLDSDGSFFLYSKLTVDKSRWQQGNVFSCSVMHEALHNHYTQKSLSLSPG

SEQ ID NO: 2 - protein, 449 aa, synthetic construct
  REGION 1..449: note = Heavy chain of Trastuzumab (humanized IgG1 monoclonal antibody)
EVQLVESGGGLVQPGGSLRLSCAASGFNIKDTYIHWVRQAPGKGLEWVARIYPTNGYTRYADSVKGRFTISADTSKNTAYLQMNSLRAEDTAVYYCSRWGGDGFYAMDYWGQGTLVTVSSASTKGPSVFPLAPSSKSTSGGTAALGCLVKDYFPEPVTVSWNSGALTSGVHTFPAVLQSSGLYSLSSVVTVPSSSLGTQTYICNVNHKPSNTKVDKKVEPKSCDKTHTCPPCPAPELLGGPSVFLFPPKPKDTLMISRTPEVTCVVVDVSHEDPEVKFNWYVDGVEVHNAKTKPREEQYDSTYRVVSVLTVLHQDWLNGKEYKCKVSNKALPAPIEKTISKAKGQPREPQVYTLPPSREEMTKNQVSLTCLVKGFYPSDIAVEWESNGQPENNYKTTPPVLDSDGSFFLYSKLTVDKSRWQQGNVFSCSVMHEALHNHYTQKSLSLSPG

SEQ ID NO: 3 - protein, 237 aa, synthetic construct
  REGION 1..237: note = Fc region of human IgG1 antibody
IEGRMDPKSCDKTHTCPPCPAPEAEGAPSVFLFPPKPKDTLMISRTPEVTCVVVDVSHEDPEVKFNWYVDGVEVHNAKTKPREEQYDSTYRVVSVLTVLHQDWLNGKEYKCKVSNKALPAPIEKTISKAKGQPREPQVYTLPPSRDELTKNQVSLTCLVKGFYPSDIAVEWESNGQPENNYKATPPVLDSDGSFFLYSKLTVDKSRWQQGNVFSCSVMHEALHNHYTQKSLSLSPGK

SEQ ID NO: 4 - protein, 214 aa, synthetic construct
  REGION 1..214: note = Light chain of Trastuzumab (humanized IgG1 monoclonal antibody)
DIQMTQSPSSLSASVGDRVTITCRASQDVNTAVAWYQQKPGKAPKLLIYSASFLYSGVPSRFSGSRSGTDFTLTISSLQPEDFATYYCQQHYTTPPTFGQGTKVEIKRTVAAPSVFIFPPSDEQLKSGTASVVCLLNNFYPREAKVQWKVDNALQSGNSQESVTEQDSKDSTYSLSSTLTLSKADYEKHKVYACEVTHQGLSSPVTKSFNRGEC

SEQ ID NO: 5 - protein, 33 aa, synthetic construct
  REGION 1..33: note = Peptide having an affinity to Fc region of human IgG. The amino acid residue at N-terminus may be acetylated, and the amino acid residue at C-terminus may be aminated.
FNMQQQRRFYEALHDPNLNEEQRNARIRSIKDD

SEQ ID NO: 6 - protein, 33 aa, synthetic construct
  REGION 1..33: note = Peptide having an affinity to Fc region of human IgG. The amino acid residue at N-terminus may be acetylated, and the amino acid residue at C-terminus may be aminated.
FNMQQQRRFYEALHDPNLNEEQRNARIKSIRDD

SEQ ID NO: 7 - protein, 33 aa, synthetic construct
  REGION 1..33: note = Peptide having an affinity to Fc region of human IgG. The amino acid residue at N-terminus may be acetylated, and the amino acid residue at C-terminus may be aminated.
  SITE 1: note = MISC_FEATURE - beta-alanine
XNMQQQRRFYEALHDPNLNEEQRNARIRSIRDD

SEQ ID NO: 8 - protein, 33 aa, synthetic construct
  REGION 1..33: note = Peptide having an affinity to Fc region of human IgG. The amino acid residue at N-terminus may be acetylated, and the amino acid residue at C-terminus may be aminated.
FNMQQQRRFYEALHDPNLNEEQRNAKIKSIKDD

SEQ ID NO: 9 - protein, 25 aa, synthetic construct
  REGION 1..25: note = Peptide having an affinity to Fc region of human IgG. The amino acid residue at N-terminus may be acetylated, and the amino acid residue at C-terminus may be aminated.
EQQNAFYEILHLPNEEQRGGGGSCG

SEQ ID NO: 10 - protein, 7 aa, synthetic construct
  REGION 1..7: note = Model for peptide drug
HHHHHHG

SEQ ID NO: 11 - protein, 33 aa, synthetic construct
  REGION 1..33: note = Peptide having an affinity to Fc region of human IgG. The amino acid residue at N-terminus may be acetylated, and the amino acid residue at C-terminus may be aminated.
FNMQQQRRFYEALHDPNLNEEQRNARIRSIRDD

SEQ ID NO: 12 - protein, 34 aa, synthetic construct
  REGION 1..34: note = Peptide having an affinity to Fc region of human IgG. The amino acid residue at N-terminus may be acetylated, and the amino acid residue at C-terminus may be aminated.
FNMQCQRRFYEALHDPNLNEEQRNARIRSIRDDC

SEQ ID NO: 13 - protein, 33 aa, synthetic construct; identical to SEQ ID NO: 7
  REGION 1..33: note = Peptide having an affinity to Fc region of human IgG. The amino acid residue at N-terminus may be acetylated, and the amino acid residue at C-terminus may be aminated.
  SITE 1: note = MISC_FEATURE - beta-alanine

SEQ ID NO: 14 - protein, 34 aa, synthetic construct
  REGION 1..34: note = Peptide having an affinity to Fc region of human IgG. The amino acid residue at N-terminus may be acetylated, and the amino acid residue at C-terminus may be aminated.
  SITE 1: note = MISC_FEATURE - beta-alanine
XNMQCQRRFYEALHDPNLNEEQRNARIRSIRDDC

SEQ ID NO: 15 - protein, 17 aa, synthetic construct
  REGION 1..17: note = Peptide having an affinity to Fc region of human IgG. The amino acid residue at N-terminus may be acetylated, the amino acid residue at C-terminus may be aminated and two cysteine residues may be linked by disulfide bridge.
  SITE 1: note = MISC_FEATURE - absent, or arginine
  SITE 2: note = MISC_FEATURE - absent, or glycine
  SITE 3: note = MISC_FEATURE - absent, aspartic acid, or asparagine
  SITE 5: note = MISC_FEATURE - alanine
  SITE 6: note = MISC_FEATURE - tyrosine, tryptophan, or histidine
  SITE 7: note = MISC_FEATURE - histidine, phenylalanine, tyrosine, tryptophan, arginine, or glycine
  SITE 8: note = MISC_FEATURE - lysine
  SITE 9: note = MISC_FEATURE - glycine, serine, asparagine, glutamine, aspartic acid, glutamic acide, phenylalanine, tyrosine, tryptophan, histidine, threonine, leucine, alanine, valine, isoleucine, or arginine
  SITE 10: note = MISC_FEATURE - glutamine, glutamic acid, asparagine, or aspartic acid
  SITE 15: note = MISC_FEATURE - absent, or threonine
  SITE 16: note = MISC_FEATURE - absent, or tyrosine
  SITE 17: note = MISC_FEATURE - absent, or histidine
XXXCXXXXXXIIWCXXX

SEQ ID NO: 16 - protein, 17 aa, synthetic construct
  REGION 1..17: note = Peptide having an affinity to Fc region of human IgG. The amino acid residue at N-terminus may be acetylated, the amino acid residue at C-terminus may be aminated and two cysteine residues may be linked by disulfide bridge.
  SITE 1: note = MISC_FEATURE - absent, or arginine
  SITE 2: note = MISC_FEATURE - absent, or glycine
  SITE 3: note = MISC_FEATURE - absent, aspartic acid, or asparagine
  SITE 5: note = MISC_FEATURE - alanine
  SITE 6: note = MISC_FEATURE - tyrosine, tryptophan, or histidine
  SITE 7: note = MISC_FEATURE - histidine, phenylalanine, tyrosine, tryptophan, arginine, or glycine
  SITE 8: note = MISC_FEATURE - lysine
  SITE 9: note = MISC_FEATURE - glycine, serine, asparagine, glutamine, aspartic acid, glutamic acide, phenylalanine, tyrosine, tryptophan, histidine, threonine, leucine, alanine, valine, isoleucine, or arginine
  SITE 10: note = MISC_FEATURE - glutamine, glutamic acid, asparagine, or aspartic acid
  SITE 15: note = MISC_FEATURE - absent, or threonine
  SITE 16: note = MISC_FEATURE - absent, or tyrosine
  SITE 17: note = MISC_FEATURE - absent, or histidine
XXXCXXXXXXIVWCXXX

SEQ ID NO: 17 - protein, 17 aa, synthetic construct
  REGION 1..17: note = Peptide having an affinity to Fc region of human IgG. The amino acid residue at N-terminus may be acetylated, the amino acid residue at C-terminus may be aminated and two cysteine residues may be linked by disulfide bridge.
  SITE 1: note = MISC_FEATURE - absent, or arginine
  SITE 2: note = MISC_FEATURE - absent, or glycine
  SITE 3: note = MISC_FEATURE - absent, aspartic acid, or asparagine
  SITE 5: note = MISC_FEATURE - alanine
  SITE 6: note = MISC_FEATURE - tyrosine, tryptophan, or histidine
  SITE 7: note = MISC_FEATURE - histidine, phenylalanine, tyrosine, tryptophan, arginine, or glycine
  SITE 8: note = MISC_FEATURE - lysine
  SITE 9: note = MISC_FEATURE - glycine, serine, asparagine, glutamine, aspartic acid, glutamic acide, phenylalanine, tyrosine, tryptophan, histidine, threonine, leucine, alanine, valine, isoleucine, or arginine
  SITE 10: note = MISC_FEATURE - glutamine, glutamic acid, asparagine, or aspartic acid
  SITE 15: note = MISC_FEATURE - absent, or threonine
  SITE 16: note = MISC_FEATURE - absent, or tyrosine
  SITE 17: note = MISC_FEATURE - absent, or histidine
XXXCXXXXXXVVWCXXX

SEQ ID NO: 18 - protein, 17 aa, synthetic construct
  REGION 1..17: note = Peptide having an affinity to Fc region of human IgG. The amino acid residue at N-terminus may be acetylated, the amino acid residue at C-terminus may be aminated and two cysteine residues may be linked by disulfide bridge.
  SITE 1: note = MISC_FEATURE - absent, or arginine
  SITE 2: note = MISC_FEATURE - absent, or glycine
  SITE 3: note = MISC_FEATURE - absent, aspartic acid, or asparagine
  SITE 5: note = MISC_FEATURE - alanine
  SITE 6: note = MISC_FEATURE - tyrosine, tryptophan, or histidine
  SITE 7: note = MISC_FEATURE - histidine, phenylalanine, tyrosine, tryptophan, arginine, or glycine
  SITE 8: note = MISC_FEATURE - lysine
  SITE 9: note = MISC_FEATURE - glycine, serine, asparagine, glutamine, aspartic acid, glutamic acide, phenylalanine, tyrosine, tryptophan, histidine, threonine, leucine, alanine, valine, isoleucine, or arginine
  SITE 10: note = MISC_FEATURE - glutamine, glutamic acid, asparagine, or aspartic acid
  SITE 15: note = MISC_FEATURE - absent, or threonine
  SITE 16: note = MISC_FEATURE - absent, or tyrosine
  SITE 17: note = MISC_FEATURE - absent, or histidine
XXXCXXXXXXAVWCXXX

SEQ ID NO: 19 - protein, 17 aa, synthetic construct
  REGION 1..17: note = Peptide having an affinity to Fc region of human IgG. The amino acid residue at N-terminus may be acetylated, the amino acid residue at C-terminus may be aminated and two cysteine residues may be linked by disulfide bridge.
  SITE 1: note = MISC_FEATURE - absent, or arginine
  SITE 2: note = MISC_FEATURE - absent, or glycine
  SITE 3: note = MISC_FEATURE - absent, aspartic acid, or asparagine
  SITE 5: note = MISC_FEATURE - alanine
  SITE 6: note = MISC_FEATURE - tyrosine, tryptophan, or histidine
  SITE 7: note = MISC_FEATURE - histidine, phenylalanine, tyrosine, tryptophan, arginine, or glycine
  SITE 8: note = MISC_FEATURE - lysine
  SITE 9: note = MISC_FEATURE - glycine, serine, asparagine, glutamine, aspartic acid, glutamic acide, phenylalanine, tyrosine, tryptophan, histidine, threonine, leucine, alanine, valine, isoleucine, or arginine
  SITE 10: note = MISC_FEATURE - glutamine, glutamic acid, asparagine, or aspartic acid
  SITE 15: note = MISC_FEATURE - absent, or threonine
  SITE 16: note = MISC_FEATURE - absent, or tyrosine
  SITE 17: note = MISC_FEATURE - absent, or histidine
XXXCXXXXXXLLWCXXX

SEQ ID NO: 20 - protein, 17 aa, synthetic construct
  REGION 1..17: note = Peptide having an affinity to Fc region of human IgG. The amino acid residue at N-terminus may be acetylated, the amino acid residue at C-terminus may be aminated and two cysteine residues may be linked by disulfide bridge.
  SITE 1: note = MISC_FEATURE - absent, or arginine
  SITE 2: note = MISC_FEATURE - absent, or glycine
  SITE 3: note = MISC_FEATURE - absent, aspartic acid, or asparagine
  SITE 5: note = MISC_FEATURE - alanine
  SITE 6: note = MISC_FEATURE - tyrosine, tryptophan, or histidine
  SITE 7: note = MISC_FEATURE - histidine, phenylalanine, tyrosine, tryptophan, arginine, or glycine
  SITE 8: note = MISC_FEATURE - lysine
  SITE 9: note = MISC_FEATURE - glycine, serine, asparagine, glutamine, aspartic acid, glutamic acide, phenylalanine, tyrosine, tryptophan, histidine, threonine, leucine, alanine, valine, isoleucine, or arginine
  SITE 10: note = MISC_FEATURE - glutamine, glutamic acid, asparagine, or aspartic acid
  SITE 15: note = MISC_FEATURE - absent, or threonine
  SITE 16: note = MISC_FEATURE - absent, or tyrosine
  SITE 17: note = MISC_FEATURE - absent, or histidine
XXXCXXXXXXLIWCXXX

SEQ ID NO: 21 - protein, 17 aa, synthetic construct
  REGION 1..17: note = Peptide having an affinity to Fc region of human IgG. The amino acid residue at N-terminus may be acetylated, the amino acid residue at C-terminus may be aminated and two cysteine residues may be linked by disulfide bridge.
  SITE 1: note = MISC_FEATURE - absent, or arginine
  SITE 2: note = MISC_FEATURE - absent, or glycine
  SITE 3: note = MISC_FEATURE - absent, aspartic acid, or asparagine
  SITE 5: note = MISC_FEATURE - alanine
  SITE 6: note = MISC_FEATURE - tyrosine, tryptophan, or histidine
  SITE 7: note = MISC_FEATURE - histidine, phenylalanine, tyrosine, tryptophan, arginine, or glycine
  SITE 8: note = MISC_FEATURE - lysine
  SITE 9: note = MISC_FEATURE - glycine, serine, asparagine, glutamine, aspartic acid, glutamic acide, phenylalanine, tyrosine, tryptophan, histidine, threonine, leucine, alanine, valine, isoleucine, or arginine
  SITE 10: note = MISC_FEATURE - glutamine, glutamic acid, asparagine, or aspartic acid
  SITE 15: note = MISC_FEATURE - absent, or threonine
  SITE 16: note = MISC_FEATURE - absent, or tyrosine
  SITE 17: note = MISC_FEATURE - absent, or histidine
XXXCXXXXXXLVFCXXX

SEQ ID NO: 22 - protein, 17 aa, synthetic construct
  REGION 1..17: note = Peptide having an affinity to Fc region of human IgG. The amino acid residue at N-terminus may be acetylated, the amino acid residue at C-terminus may be aminated and two cysteine residues may be linked by disulfide bridge.
  SITE 1: note = MISC_FEATURE - absent, or arginine
  SITE 2: note = MISC_FEATURE - absent, or glycine
  SITE 3: note = MISC_FEATURE - absent, aspartic acid, or asparagine
  SITE 5: note = MISC_FEATURE - alanine
  SITE 6: note = MISC_FEATURE - tyrosine, tryptophan, or histidine
  SITE 7: note = MISC_FEATURE - histidine, phenylalanine, tyrosine, tryptophan, arginine, or glycine
  SITE 8: note = MISC_FEATURE - lysine
  SITE 9: note = MISC_FEATURE - glycine, serine, asparagine, glutamine, aspartic acid, glutamic acide, phenylalanine, tyrosine, tryptophan, histidine, threonine, leucine, alanine, valine, isoleucine, or arginine
  SITE 10: note = MISC_FEATURE - glutamine, glutamic acid, asparagine, or aspartic acid
  SITE 15: note = MISC_FEATURE - absent, or threonine
  SITE 16: note = MISC_FEATURE - absent, or tyrosine
  SITE 17: note = MISC_FEATURE - absent, or histidine
XXXCXXXXXXQVWCXXX

SEQ ID NO: 23 - protein, 17 aa, synthetic construct
  REGION 1..17: note = Peptide having an affinity to Fc region of human IgG. The amino acid residue at N-terminus may be acetylated, the amino acid residue at C-terminus may be aminated and two cysteine residues may be linked by disulfide bridge.
  SITE 1: note = MISC_FEATURE - absent, or arginine
  SITE 2: note = MISC_FEATURE - absent, or glycine
  SITE 3: note = MISC_FEATURE - absent, aspartic acid, or asparagine
  SITE 5: note = MISC_FEATURE - alanine
  SITE 6: note = MISC_FEATURE - tyrosine, tryptophan, or histidine
  SITE 7: note = MISC_FEATURE - histidine, phenylalanine, tyrosine, tryptophan, arginine, or glycine
  SITE 8: note = MISC_FEATURE - lysine
  SITE 9: note = MISC_FEATURE - glycine, serine, asparagine, glutamine, aspartic acid, glutamic acide, phenylalanine, tyrosine, tryptophan, histidine, threonine, leucine, alanine, valine, isoleucine, or arginine
  SITE 10: note = MISC_FEATURE - glutamine, glutamic acid, asparagine, or aspartic acid
  SITE 15: note = MISC_FEATURE - absent, or threonine
  SITE 16: note = MISC_FEATURE - absent, or tyrosine
  SITE 17: note = MISC_FEATURE - absent, or histidine
XXXCXXXXXXEVWCXXX

SEQ ID NO: 24 - protein, 17 aa, synthetic construct
  REGION 1..17: note = Peptide having an affinity to Fc region of human IgG. The amino acid residue at N-terminus may be acetylated, the amino acid residue at C-terminus may be aminated and two cysteine residues may be linked by disulfide bridge.
  SITE 1: note = MISC_FEATURE - absent, or arginine
  SITE 2: note = MISC_FEATURE - absent, or glycine
  SITE 3: note = MISC_FEATURE - absent, aspartic acid, or asparagine
  SITE 5: note = MISC_FEATURE - alanine
  SITE 6: note = MISC_FEATURE - tyrosine, tryptophan, or histidine
  SITE 7: note = MISC_FEATURE - histidine, phenylalanine, tyrosine, tryptophan, arginine, or glycine
  SITE 8: note = MISC_FEATURE - lysine
  SITE 9: note = MISC_FEATURE - glycine, serine, asparagine, glutamine, aspartic acid, glutamic acide, phenylalanine, tyrosine, tryptophan, histidine, threonine, leucine, alanine, valine, isoleucine, or arginine
  SITE 10: note = MISC_FEATURE - glutamine, glutamic acid, asparagine, or aspartic acid
  SITE 15: note = MISC_FEATURE - absent, or threonine
  SITE 16: note = MISC_FEATURE - absent, or tyrosine
  SITE 17: note = MISC_FEATURE - absent, or histidine
XXXCXXXXXXLVWCXXX

SEQ ID NO: 25 - protein, 12 aa, synthetic construct
  REGION 1..12: note = Peptide having an affinity to CH2 region of human IgG
EPIHRSTLTALL

SEQ ID NO: 26 - protein, 10 aa, synthetic construct
  REGION 1..10: note = Peptide having an affinity to Fc region of human IgG
FARLVSSIRY

SEQ ID NO: 27 - protein, 10 aa, synthetic construct
  REGION 1..10: note = Peptide having an affinity to Fc region of human IgG
FGRLVSSIRY

SEQ ID NO: 28 - protein, 10 aa, synthetic construct
  REGION 1..10: note = Peptide having an affinity to Fc region of human IgG
TWKTSRISIF

SEQ ID NO: 29 - protein, 4 aa, synthetic construct
  REGION 1..4: note = Peptide having an affinity to specific region of human IgG
QSYP

SEQ ID NO: 30 - protein, 6 aa, synthetic construct
  REGION 1..6: note = Peptide having an affinity to Fc region of human IgG
HWRGWV

SEQ ID NO: 31 - protein, 6 aa, synthetic construct
  REGION 1..6: note = Peptide having an affinity to Fc region of human IgG
HYFKFD

SEQ ID NO: 32 - protein, 6 aa, synthetic construct
  REGION 1..6: note = Peptide having an affinity to Fc region of human IgG
HFRRHL

SEQ ID NO: 33 - protein, 4 aa, synthetic construct
  REGION 1..4: note = Peptide having an affinity to Fc region of human IgG
DAAG

SEQ ID NO: 34 - protein, 8 aa, synthetic construct
  REGION 1..8: note = Peptide having an affinity to Fc region of human IgG
NARKFYKG

SEQ ID NO: 35 - protein, 8 aa, synthetic construct
  REGION 1..8: note = Peptide having an affinity to Fc region of human IgG
NKFRGKYK

SEQ ID NO: 36 - protein, 34 aa, synthetic construct
  REGION 1..34: note = Phenylalanine residue at N-terminus may be acetylated and two cysteine residues may be linked by disulfide bridge
FNMQCQRRFYEALHDPNLNEEQRNAKIKSIRDDC

SEQ ID NO: 37 - protein, 34 aa, synthetic construct
  REGION 1..34: note = Lysine residue at N-terminus may be acetylated and two cysteine residues may be linked by disulfide bridge
KNMQCQRRFYEALHDPNLNEEQRNARIRSIRDDC

SEQ ID NO: 38 - protein, 34 aa, synthetic construct
  REGION 1..34: note = Phenylalanine residue at N-terminus may be acetylated and two cysteine residues may be linked by disulfide bridge
FNMQCQKRFYEALHDPNLNEEQRNARIRSIRDDC

SEQ ID NO: 39 - protein, 34 aa, synthetic construct
  REGION 1..34: note = Phenylalanine residue at N-terminus may be acetylated and two cysteine residues may be linked by disulfide bridge
FNMQCQRRFYEAKHDPNLNEEQRNARIRSIRDDC

SEQ ID NO: 40 - protein, 34 aa, synthetic construct
  REGION 1..34: note = Phenylalanine residue at N-terminus may be acetylated and two cysteine residues may be linked by disulfide bridge
FNMQCQRRFYEALHDPNLNEEQRKARIRSIRDDC

SEQ ID NO: 41 - protein, 34 aa, synthetic construct
  REGION 1..34: note = Phenylalanine residue at N-terminus may be acetylated and two cysteine residues may be linked by disulfide bridge
FNMQCQRRFYEALHDPNLNKEQRNARIRSIRDDC

SEQ ID NO: 42 - protein, 34 aa, synthetic construct
  REGION 1..34: note = Phenylalanine residue at N-terminus may be acetylated and two cysteine residues may be linked by disulfide bridge
FNMQCQRRFYEALHDPNLNEEQRNARIRSIKDDC

SEQ ID NO: 43 - protein, 34 aa, synthetic construct
  REGION 1..34: note = Phenylalanine residue at N-terminus may be acetylated and two cysteine residues may be linked by disulfide bridge
FNKQCQRRFYEALHDPNLNEEQRNARIRSIRDDC

SEQ ID NO: 44 - protein, 34 aa, synthetic construct
  REGION 1..34: note = Phenylalanine residue at N-terminus may be acetylated and two cysteine residues may be linked by disulfide bridge
FNMQCKRRFYEALHDPNLNEEQRNARIRSIRDDC

SEQ ID NO: 45 - protein, 34 aa, synthetic construct
  REGION 1..34: note = Phenylalanine residue at N-terminus may be acetylated and two cysteine residues may be linked by disulfide bridge
FNMQCQRRFYEALHDPNLNEEQRNARIRSIRKDC

SEQ ID NO: 46 - protein, 17 aa, synthetic construct
  REGION 1..17: note = Peptide having an affinity to Fc region of human IgG. The amino acid residue at N-terminus may be acetylated, the amino acid residue at C-terminus may be aminated and two cysteine residues may be linked by disulfide bridge.
RGNCAYHKGQIIWCTYH

SEQ ID NO: 47 - protein, 17 aa, synthetic construct
  REGION 1..17: note = Peptide having an affinity to Fc region of human IgG. The amino acid residue at N-terminus may be acetylated, the amino acid residue at C-terminus may be aminated and two cysteine residues may be linked by disulfide bridge.
RGNCAYHKGQIVWCTYH

SEQ ID NO: 48 - protein, 17 aa, synthetic construct
  REGION 1..17: note = Peptide having an affinity to Fc region of human IgG. The amino acid residue at N-terminus may be acetylated, the amino acid residue at C-terminus may be aminated and two cysteine residues may be linked by disulfide bridge.
RGNCAYHKGQVVWCTYH

SEQ ID NO: 49 - protein, 17 aa, synthetic construct
  REGION 1..17: note = Peptide having an affinity to Fc region of human IgG. The amino acid residue at N-terminus may be acetylated, the amino acid residue at C-terminus may be aminated and two cysteine residues may be linked by disulfide bridge.
RGNCAYHKGQAVWCTYH

SEQ ID NO: 50 - protein, 17 aa, synthetic construct
  REGION 1..17: note = Peptide having an affinity to Fc region of human IgG. The amino acid residue at N-terminus may be acetylated, the amino acid residue at C-terminus may be aminated and two cysteine residues may be linked by disulfide bridge.
RGNCAYHKGQLLWCTYH

SEQ ID NO: 51 - protein, 17 aa, synthetic construct
  REGION 1..17: note = Peptide having an affinity to Fc region of human IgG. The amino acid residue at N-terminus may be acetylated, the amino acid residue at C-terminus may be aminated and two cysteine residues may be linked by disulfide bridge.
RGNCAYHKGQLIWCTYH

SEQ ID NO: 52 - protein, 13 aa, synthetic construct
  REGION 1..13: note = Peptide having an affinity to Fc region of human IgG. The amino acid residue at N-terminus may be acetylated, the amino acid residue at C-terminus may be aminated and two cysteine residues may be linked by disulfide bridge.
DCAYHKGQIVWCT

SEQ ID NO: 53 - protein, 13 aa, synthetic construct
  REGION 1..13: note = Peptide having an affinity to Fc region of human IgG. The amino acid residue at N-terminus may be acetylated, the amino acid residue at C-terminus may be aminated and two cysteine residues may be linked by disulfide bridge.
DCAYHKGQVVWCT

SEQ ID NO: 54 - protein, 13 aa, synthetic construct
  REGION 1..13: note = Peptide having an affinity to Fc region of human IgG. The amino acid residue at N-terminus may be acetylated, the amino acid residue at C-terminus may be aminated and two cysteine residues may be linked by disulfide bridge.
DCAYHKGQAVWCT

SEQ ID NO: 55 - protein, 17 aa, synthetic construct
  REGION 1..17: note = eptide having an affinity to Fc region of human IgG. The amino acid residue at N-terminus may be acetylated, the amino acid residue at C-terminus may be aminated and two cysteine residues may be linked by disulfide bridge.
RGNCAYHKSQIIWCTYH

SEQ ID NO: 56 - protein, 17 aa, synthetic construct
  REGION 1..17: note = Peptide having an affinity to Fc region of human IgG. The amino acid residue at N-terminus may be acetylated, the amino acid residue at C-terminus may be aminated and two cysteine residues may be linked by disulfide bridge.
RGNCAYHKNQIIWCTYH

SEQ ID NO: 57 - protein, 17 aa, synthetic construct
  REGION 1..17: note = Peptide having an affinity to Fc region of human IgG. The amino acid residue at N-terminus may be acetylated, the amino acid residue at C-terminus may be aminated and two cysteine residues may be linked by disulfide bridge.
RGNCAYHKDQIIWCTYH

SEQ ID NO: 58 - protein, 17 aa, synthetic construct
  REGION 1..17: note = Peptide having an affinity to Fc region of human IgG. The amino acid residue at N-terminus may be acetylated, the amino acid residue at C-terminus may be aminated and two cysteine residues may be linked by disulfide bridge.
RGNCAYHKQQIIWCTYH

SEQ ID NO: 59 - protein, 17 aa, synthetic construct
  REGION 1..17: note = Peptide having an affinity to Fc region of human IgG. The amino acid residue at N-terminus may be acetylated, the amino acid residue at C-terminus may be aminated and two cysteine residues may be linked by disulfide bridge.
RGNCAYHKEQIIWCTYH

SEQ ID NO: 60 - protein, 17 aa, synthetic construct
  REGION 1..17: note = Peptide having an affinity to Fc region of human IgG. The amino acid residue at N-terminus may be acetylated, the amino acid residue at C-terminus may be aminated and two cysteine residues may be linked by disulfide bridge.
RGNCAYHKFQIIWCTYH

SEQ ID NO: 61 - protein, 17 aa, synthetic construct
  REGION 1..17: note = Peptide having an affinity to Fc region of human IgG. The amino acid residue at N-terminus may be acetylated, the amino acid residue at C-terminus may be aminated and two cysteine residues may be linked by disulfide bridge.
RGNCAYHKYQIIWCTYH

SEQ ID NO: 62 - protein, 17 aa, synthetic construct
  REGION 1..17: note = Peptide having an affinity to Fc region of human IgG. The amino acid residue at N-terminus may be acetylated, the amino acid residue at C-terminus may be aminated and two cysteine residues may be linked by disulfide bridge.
RGNCAYHKWQIIWCTYH

SEQ ID NO: 63 - protein, 17 aa, synthetic construct
  REGION 1..17: note = Peptide having an affinity to Fc region of human IgG. The amino acid residue at N-terminus may be acetylated, the amino acid residue at C-terminus may be aminated and two cysteine residues may be linked by disulfide bridge.
RGNCAYHKHQIIWCTYH

SEQ ID NO: 64 - protein, 17 aa, synthetic construct
  REGION 1..17: note = Peptide having an affinity to Fc region of human IgG. The amino acid residue at N-terminus may be acetylated, the amino acid residue at C-terminus may be aminated and two cysteine residues may be linked by disulfide bridge.
RGNCAYHKTQIIWCTYH

SEQ ID NO: 65 - protein, 17 aa, synthetic construct
  REGION 1..17: note = Peptide having an affinity to Fc region of human IgG. The amino acid residue at N-terminus may be acetylated, the amino acid residue at C-terminus may be aminated and two cysteine residues may be linked by disulfide bridge.
RGNCAYHKLQIIWCTYH

SEQ ID NO: 66 - protein, 11 aa, synthetic construct
  REGION 1..11: note = Peptide having an affinity to Fc region of human IgG. The amino acid residue at N-terminus may be acetylated, the amino acid residue at C-terminus may be aminated and two cysteine residues may be linked by disulfide bridge.
CAYHKLQIVWC

SEQ ID NO: 67 - protein, 11 aa, synthetic construct
  REGION 1..11: note = Peptide having an affinity to Fc region of human IgG. The amino acid residue at N-terminus may be acetylated, the amino acid residue at C-terminus may be aminated and two cysteine residues may be linked by disulfide bridge.
CAYHKLQLIWC

SEQ ID NO: 68 - protein, 11 aa, synthetic construct
  REGION 1..11: note = Peptide having an affinity to Fc region of human IgG. The amino acid residue at N-terminus may be acetylated, the amino acid residue at C-terminus may be aminated and two cysteine residues may be linked by disulfide bridge.
CAYHKSQIVWC

SEQ ID NO: 69 - protein, 17 aa, synthetic construct
  REGION 1..17: note = Peptide having an affinity to Fc region of human IgG. The amino acid residue at N-terminus may be acetylated, the amino acid residue at C-terminus may be aminated and two cysteine residues may be linked by disulfide bridge.
RGNCAYHKGQLVFCTYH

SEQ ID NO: 70 - protein, 17 aa, synthetic construct
  REGION 1..17: note = Peptide having an affinity to Fc region of human IgG. The amino acid residue at N-terminus may be acetylated, the amino acid residue at C-terminus may be aminated and two cysteine residues may be linked by disulfide bridge.
RGNCAYHKGQQVWCTYH

SEQ ID NO: 71 - protein, 17 aa, synthetic construct
  REGION 1..17: note = Peptide having an affinity to Fc region of human IgG. The amino acid residue at N-terminus may be acetylated, the amino acid residue at C-terminus may be aminated and two cysteine residues may be linked by disulfide bridge.
RGNCAYHKGQEVWCTYH

SEQ ID NO: 72 - protein, 11 aa, synthetic construct
  REGION 1..11: note = Peptide having an affinity to Fc region of human IgG. The amino acid residue at N-terminus may be acetylated, the amino acid residue at C-terminus may be aminated and two cysteine residues may be linked by disulfide bridge.
CAYHKGQLVWC

SEQ ID NO: 73 - protein, 17 aa, synthetic construct
  REGION 1..17: note = Peptide having an affinity to Fc region of human IgG. The amino acid residue at N-terminus may be acetylated, the amino acid residue at C-terminus may be aminated and two cysteine residues may be linked by disulfide bridge.
RGNCAYHKAQLVWCTYH

SEQ ID NO: 74 - protein, 17 aa, synthetic construct
  REGION 1..17: note = Peptide having an affinity to Fc region of human IgG. The amino acid residue at N-terminus may be acetylated, the amino acid residue at C-terminus may be aminated and two cysteine residues may be linked by disulfide bridge.
RGNCAYHKVQLVWCTYH

SEQ ID NO: 75 - protein, 17 aa, synthetic construct
  REGION 1..17: note = Peptide having an affinity to Fc region of human IgG. The amino acid residue at N-terminus may be acetylated, the amino acid residue at C-terminus may be aminated and two cysteine residues may be linked by disulfide bridge.
RGNCAYHKLQLVWCTYH

SEQ ID NO: 76 - protein, 17 aa, synthetic construct
  REGION 1..17: note = Peptide having an affinity to Fc region of human IgG. The amino acid residue at N-terminus may be acetylated, the amino acid residue at C-terminus may be aminated and two cysteine residues may be linked by disulfide bridge.
RGNCAYHKIQLVWCTYH

SEQ ID NO: 77 - protein, 17 aa, synthetic construct
  REGION 1..17: note = Peptide having an affinity to Fc region of human IgG. The amino acid residue at N-terminus may be acetylated, the amino acid residue at C-terminus may be aminated and two cysteine residues may be linked by disulfide bridge.
RGNCAYHKSQLVWCTYH

SEQ ID NO: 78 - protein, 17 aa, synthetic construct
  REGION 1..17: note = Peptide having an affinity to Fc region of human IgG. The amino acid residue at N-terminus may be acetylated, the amino acid residue at C-terminus may be aminated and two cysteine residues may be linked by disulfide bridge.
RGNCAYHKTQLVWCTYH

SEQ ID NO: 79 - protein, 17 aa, synthetic construct
  REGION 1..17: note = Peptide having an affinity to Fc region of human IgG. The amino acid residue at N-terminus may be acetylated, the amino acid residue at C-terminus may be aminated and two cysteine residues may be linked by disulfide bridge.
RGNCAYHKNQLVWCTYH

SEQ ID NO: 80 - protein, 17 aa, synthetic construct
  REGION 1..17: note = Peptide having an affinity to Fc region of human IgG. The amino acid residue at N-terminus may be acetylated, the amino acid residue at C-terminus may be aminated and two cysteine residues may be linked by disulfide bridge.
RGNCAYHKDQLVWCTYH

SEQ ID NO: 81 - protein, 17 aa, synthetic construct
  REGION 1..17: note = Peptide having an affinity to Fc region of human IgG. The amino acid residue at N-terminus may be acetylated, the amino acid residue at C-terminus may be aminated and two cysteine residues may be linked by disulfide bridge.
RGNCAYHKQQLVWCTYH

SEQ ID NO: 82 - protein, 17 aa, synthetic construct
  REGION 1..17: note = Peptide having an affinity to Fc region of human IgG. The amino acid residue at N-terminus may be acetylated, the amino acid residue at C-terminus may be aminated and two cysteine residues may be linked by disulfide bridge.
RGNCAYHKEQLVWCTYH

SEQ ID NO: 83 - protein, 17 aa, synthetic construct
  REGION 1..17: note = Peptide having an affinity to Fc region of human IgG. The amino acid residue at N-terminus may be acetylated, the amino acid residue at C-terminus may be aminated and two cysteine residues may be linked by disulfide bridge.
RGNCAYHKFQLVWCTYH

SEQ ID NO: 84 - protein, 17 aa, synthetic construct
  REGION 1..17: note = Peptide having an affinity to Fc region of human IgG. The amino acid residue at N-terminus may be acetylated, the amino acid residue at C-terminus may be aminated and two cysteine residues may be linked by disulfide bridge.
RGNCAYHKRQLVWCTYH

SEQ ID NO: 85 - protein, 17 aa, synthetic construct
  REGION 1..17: note = Peptide having an affinity to Fc region of human IgG. The amino acid residue at N-terminus may be acetylated, the amino acid residue at C-terminus may be aminated and two cysteine residues may be linked by disulfide bridge.
RGNCAYHKHQLVWCTYH

SEQ ID NO: 86 - protein, 17 aa, synthetic construct
  REGION 1..17: note = Peptide having an affinity to Fc region of human IgG. The amino acid residue at N-terminus may be acetylated, the amino acid residue at C-terminus may be aminated and two cysteine residues may be linked by disulfide bridge.
RGNCAYHKWQLVWCTYH

SEQ ID NO: 87 - protein, 17 aa, synthetic construct
  REGION 1..17: note = Peptide having an affinity to Fc region of human IgG. The amino acid residue at N-terminus may be acetylated, the amino acid residue at C-terminus may be aminated and two cysteine residues may be linked by disulfide bridge.
RGNCAYHKYQLVWCTYH

SEQ ID NO: 88 - protein, 17 aa, synthetic construct
  REGION 1..17: note = Peptide having an affinity to Fc region of human IgG. The amino acid residue at N-terminus may be acetylated, the amino acid residue at C-terminus may be aminated and two cysteine residues may be linked by disulfide bridge.
RGNCAYFKGQLVWCTYH

SEQ ID NO: 89 - protein, 17 aa, synthetic construct
  REGION 1..17: note = Peptide having an affinity to Fc region of human IgG. The amino acid residue at N-terminus may be acetylated, the amino acid residue at C-terminus may be aminated and two cysteine residues may be linked by disulfide bridge.
RGNCAYYKGQLVWCTYH

SEQ ID NO: 90 - protein, 17 aa, synthetic construct
  REGION 1..17: note = Peptide having an affinity to Fc region of human IgG. The amino acid residue at N-terminus may be acetylated, the amino acid residue at C-terminus may be aminated and two cysteine residues may be linked by disulfide bridge.
RGNCAYWKGQLVWCTYH

SEQ ID NO: 91 - protein, 17 aa, synthetic construct
  REGION 1..17: note = Peptide having an affinity to Fc region of human IgG. The amino acid residue at N-terminus may be acetylated, the amino acid residue at C-terminus may be aminated and two cysteine residues may be linked by disulfide bridge.
RGNCAYRKGQLVWCTYH

SEQ ID NO: 92 - protein, 17 aa, synthetic construct
  REGION 1..17: note = Peptide having an affinity to Fc region of human IgG. The amino acid residue at N-terminus may be acetylated, the amino acid residue at C-terminus may be aminated and two cysteine residues may be linked by disulfide bridge.
RGNCAYGKGQLVWCTYH

SEQ ID NO: 93 - protein, 12 aa, synthetic construct
  REGION 1..12: note = Peptide having an affinity to Fc region of human IgG. The amino acid residue at N-terminus may be acetylated, the amino acid residue at C-terminus may be aminated and two cysteine residues may be linked by disulfide bridge.
DCAYHKGQLVWC

SEQ ID NO: 94 - protein, 12 aa, synthetic construct
  REGION 1..12: note = Peptide having an affinity to Fc region of human IgG. The amino acid residue at N-terminus may be acetylated, the amino acid residue at C-terminus may be aminated and two cysteine residues may be linked by disulfide bridge.
NCAYHKGQLVWC

SEQ ID NO: 95 - protein, 12 aa, synthetic construct
  REGION 1..12: note = Peptide having an affinity to Fc region of human IgG. The amino acid residue at N-terminus may be acetylated, the amino acid residue at C-terminus may be aminated and two cysteine residues may be linked by disulfide bridge.
CAYHKGQLVWCT

SEQ ID NO: 96 - protein, 11 aa, synthetic construct
  REGION 1..11: note = Peptide having an affinity to Fc region of human IgG. The amino acid residue at N-terminus may be acetylated, the amino acid residue at C-terminus may be aminated and two cysteine residues may be linked by disulfide bridge.
CAYHKSQLVWC

SEQ ID NO: 97 - protein, 28 aa, synthetic construct
  REGION 1..28: note = Peptide having an affinity to Fc region of human IgG. The amino acid residue at N-terminus may be acetylated, and the amino acid residue at C-terminus may be aminated.
NMQQQRRFYEALHDPNLEEQRNARIRSI

SEQ ID NO: 98 - protein, 33 aa, synthetic construct
  REGION 1..33: note = Peptide having an affinity to Fc region of human IgG. The amino acid residue at N-terminus may be acetylated, and the amino acid residue at C-terminus may be aminated.
FNMQQQRRFYEALHDPNLNKEQRNARIRSIRDD

SEQ ID NO: 99 - protein, 16 aa, synthetic construct
  REGION 1..16: note = Peptide having an affinity to Fc region of human IgG. The amino acid residue at N-terminus may be acetylated, the amino acid residue at C-terminus may be aminated and two cysteine residues may be linked by disulfide bridge.
GNCAYHKGQIIWCTYH

SEQ ID NO: 100 - protein, 31 aa, synthetic construct
  REGION 1..31: note = Peptide having an affinity to Fc region of human IgG. The amino acid residue at N-terminus may be acetylated, and the amino acid residue at C-terminus may be aminated.
NMQQQRRFYEALHDPNLEEQRNARIRSIKDD

SEQ ID NO: 101 - protein, 19 aa, synthetic construct
  REGION 1..19: note = Peptice fragment containing lysin residue at position 317 in human IgG
VVSVLTVLHQDWLNGKEYK

SEQ ID NO: 102 - protein, 33 aa, synthetic construct
  REGION 1..33: note = Peptice fragment containing lysin residue at position 247or 249 in denosumab
CCVECPPCPAPPVAGPSVFLFPPKPKDTLMISR

SEQ ID NO: 103 - protein, 34 aa, synthetic construct
  REGION 1..34: note = Peptice fragment containing lysin residue at position 251or 253 in dupixent
YGPPCPPCPAPEFLGGPSVFLFPPKPKDTLMISR

SEQ ID NO: 104 - protein, 447 aa, synthetic construct
  REGION 1..447: note = Amino acid sequence of heavy chain of denosumab
EVQLLESGGGLVQPGGSLRLSCAASGFTFSSYAMSWVRQAPGKGLEWVSGITGSGGSTYYADSVKGRFTISRDNSKNTLYLQMNSLRAEDTAVYYCAKDPGTTVIMSWFDPWGQGTLVTVSSASTKGPSVFPLAPCSRSTSESTAALGCLVKDYFPEPVTVSWNSGALTSGVHTFPAVLQSSGLYSLSSVVTVPSSNFGTQTYTCNVDHKPSNTKVDKTVERKCCVECPPCPAPPVAGPSVFLFPPKPKDTLMISRTPEVTCVVVDVSHEDPEVQFNWYVDGVEVHNAKTKPREEQFNSTFRVVSVLTVVHQDWLNGKEYKCKVSNKGLPAPIEKTISKTKGQPREPQVYTLPPSREEMTKNQVSLTCLVKGFYPSDIAVEWESNGQPENNYKTTPPMLDSDGSFFLYSKLTVDKSRWQQGNVFSCSVMHEALHNHYTQKSLSLSPG

SEQ ID NO: 105 - protein, 215 aa, synthetic construct
  REGION 1..215: note = Amino acid sequence of light chain of denosumab
EIVLTQSPGTLSLSPGERATLSCRASQSVRGRYLAWYQQKPGQAPRLLIYGASSRATGIPDRFSGSGSGTDFTLTISRLEPEDFAVFYCQQYGSSPRTFGQGTKVEIKRTVAAPSVFIFPPSDEQLKSGTASVVCLLNNFYPREAKVQWKVDNALQSGNSQESVTEQDSKDSTYSLSSTLTLSKADYEKHKVYACEVTHQGLSSPVTKSFNRGEC

SEQ ID NO: 106 - protein, 452 aa, synthetic construct
  REGION 1..452: note = Amino acid sequence of heavy chain of dupixent
EVQLVESGGGLEQPGGSLRLSCAGSGFTFRDYAMTWVRQAPGKGLEWVSSISGSGGNTYYADSVKGRFTISRDNSKNTLYLQMNSLRAEDTAVYYCAKDRLSITIRPRYYGLDVWGQGTTVTVSSASTKGPSVFPLAPCSRSTSESTAALGCLVKDYFPEPVTVSWNSGALTSGVHTFPAVLQSSGLYSLSSVVTVPSSSLGTKTYTCNVDHKPSNTKVDKRVESKYGPPCPPCPAPEFLGGPSVFLFPPKPKDTLMISRTPEVTCVVVDVSQEDPEVQFNWYVDGVEVHNAKTKPREEQFNSTYRVVSVLTVLHQDWLNGKEYKCKVSNKGLPSSIEKTISKAKGQPREPQVYTLPPSQEEMTKNQVSLTCLVKGFYPSDIAVEWESNGQPENNYKTTPPVLDSDGSFFLYSRLTVDKSRWQEGNVFSCSVMHEALHNHYTQKSLSLSLGK

SEQ ID NO: 107 - protein, 219 aa, synthetic construct
  REGION 1..219: note = Amino acid sequence of light chain of dupixent
DIVMTQSPLSLPVTPGEPASISCRSSQSLLYSIGYNYLDWYLQKSGQSPQLLIYLGSNRASGVPDRFSGSGSGTDFTLKISRVEAEDVGFYYCMQALQTPYTFGQGTKLEIKRTVAAPSVFIFPPSDEQLKSGTASVVCLLNNFYPREAKVQWKVDNALQSGNSQESVTEQDSKDSTYSLSSTLTLSKADYEKHKVYACEVTHQGLSSPVTKSFNRGEC

SEQ ID NO: 108 - protein, 17 aa, synthetic construct
  REGION 1..17: note = Peptide having an affinity to Fc region of human IgG. The amino acid residue at N-terminus may be acetylated, the amino acid residue at C-terminus may be aminated and two cysteine residues may be linked by disulfide bridge.
RGNCAYHEGQIIWCTYH